European Patent Application EP 4 119 133 A1, published January 18, 2023. Title: Use of glutamine synthetase for treating hyperammonemia. Applicant: Ammun Limited. Application GB 1800867.2. The sequence listing filed with the application follows.

SEQUENCE LISTING (7 sequences)

SEQ ID NO: 1 - protein, 373 aa, Homo sapiens
MTTSASSHLNKGIKQVYMSLPQGEKVQAMYIWIDGTGEGLRCKTRTLDSEPKCVEELPEWNFDGSSTLQSEGSNSDMYLVPAAMFRDPFRKDPNKLVLCEVFKYNRRPAETNLRHTCKRIMDMVSNQHPWFGMEQEYTLMGTDGHPFGWPSNGFPGPQGPYYCGVGADRAYGRDIVEAHYRACLYAGVKIAGTNAEVMPAQWEFQIGPCEGISMGDHLWVARFILHRVCEDFGVIATFDPKPIPGNWNGAGCHTNFSTKAMREENGLKYIEEAIEKLSKRHQYHIRAYDPKGGLDNARRLTGFHETSNINDFSAGVANRSASIRIPRTVGQEKKGYFEDRRPSANCDPFSVTEALIRTCLLNETGDEPFQYKN

SEQ ID NO: 2 - protein, 372 aa, Homo sapiens
TTSASSHLNKGIKQVYMSLPQGEKVQAMYIWIDGTGEGLRCKTRTLDSEPKCVEELPEWNFDGSSTLQSEGSNSDMYLVPAAMFRDPFRKDPNKLVLCEVFKYNRRPAETNLRHTCKRIMDMVSNQHPWFGMEQEYTLMGTDGHPFGWPSNGFPGPQGPYYCGVGADRAYGRDIVEAHYRACLYAGVKIAGTNAEVMPAQWEFQIGPCEGISMGDHLWVARFILHRVCEDFGVIATFDPKPIPGNWNGAGCHTNFSTKAMREENGLKYIEEAIEKLSKRHQYHIRAYDPKGGLDNARRLTGFHETSNINDFSAGVANRSASIRIPRTVGQEKKGYFEDRRPSANCDPFSVTEALIRTCLLNETGDEPFQYKN

SEQ ID NO: 3 - DNA, 1366 bp, Homo sapiens
cgagagtgggagaagagcggagcgtgtgagcagtactgcggcctcctctcctctcctaacctgctctcgcggcctacctttacccgcccgcctgctcggcgaccagaacaccttccaccatgaccacctcagcaagttcccacttaaataaaggcatcaagcaggtgtacatgtccctgcctcagggtgagaaagtccaggccatgtatatctggatcgatggtactggagaaggactgcgctgcaagacccggaccctggacagtgagcccaagtgtgtggaagagttgcctgagtggaatttcgatggctccagtactttacagtctgagggttccaacagtgacatgtatctcgtgcctgctgccatgtttcgggaccccttccgtaaggaccctaacaagctggtgttatgtgaagttttcaagtacaatcgaaggcctgcagagaccaatttgaggcacacctgtaaacggataatggacatggtgagcaaccagcacccctggtttggcatggagcaggagtataccctcatggggacagatgggcacccctttggttggccttccaacggcttcccagggccccagggtccatattactgtggtgtgggagcagacagagcctatggcagggacatcgtggaggcccattaccgggcctgcttgtatgctggagtcaagattgcggggactaatgccgaggtcatgcctgcccagtgggaatttcagattggaccttgtgaaggaatcagcatgggagatcatctctgggtggcccgtttcatcttgcatcgtgtgtgtgaagactttggagtgatagcaacctttgatcctaagcccattcctgggaactggaatggtgcaggctgccataccaacttcagcaccaaggccatgcgggaggagaatggtctgaagtacatcgaggaggccattgagaaactaagcaagcggcaccagtaccacatccgtgcctatgatcccaagggaggcctggacaatgcccgacgtctaactggattccatgaaacctccaacatcaacgacttttctggtggtgtagccaatcgtagcgccagcatacgcattccccggactgttggccaggagaagaagggttactttgaagatcgtcgcccctctgccaactgcgaccccttttcggtgacagaagccctcatccgcacgtgtcttctcaatgaaaccggcgatgagcccttccagtacaaaaattaagtggactagacctccagctgttgagcccctcctagttcttcatcccactccaactcttccccctctcccagttgtcccgattgtaactcaaagggtggaatatcaaggtcgttttttttcattcc

SEQ ID NO: 4 - protein, 388 aa, Artificial Sequence
  Modified human GS protein
MGSSHHHHHHGGGGSMTTSASSHLNKGIKQVYMSLPQGEKVQAMYIWIDGTGEGLRCKTRTLDSEPKCVEELPEWNFDGSSTLQSEGSNSDMYLVPAAMFRDPFRKDPNKLVLCEVFKYNRRPAETNLRHTCKRIMDMVSNQHPWFGMEQEYTLMGTDGHPFGWPSNGFPGPQGPYYCGVGADRAYGRDIVEAHYRACLYAGVKIAGTNAEVMPAQWEFQIGPCEGISMGDHLWVARFILHRVCEDFGVIATFDPKPIPGNWNGAGCHTNFSTKAMREENGLKYIEEAIEKLSKRHQYHIRAYDPKGGLDNARRLTGFHETSNINDFSAGVANRSASIRIPRTVGQEKKGYFEDRRPSANCDPFSVTEALIRTCLLNETGDEPFQYKN

SEQ ID NO: 5 - DNA, 1164 bp, Artificial Sequence
  pET30a+ vector, containing the gene for human GS
atgggcagcagccaccaccatcaccaccacggcggcggcggtagcatgaccacctcggcaagcagccacctgaataaaggcatcaaacaggtgtatatgtctctgccgcagggtgaaaaagttcaagccatgtacatttggatcgatggcaccggtgaaggcctgcgttgcaaaacccgcacgctggactcagaaccgaaatgtgtggaagaactgccggaatggaactttgatggtagctctacgctgcagtcggaaggcagtaattccgacatgtatctggttccggcggccatgtttcgtgatccgttccgcaaagacccgaacaaactggtgctgtgcgaagtttttaaatacaaccgtcgcccggcggaaaccaatctgcgtcatacgtgtaaacgcattatggatatggtcagcaaccagcacccgtggttcggtatggaacaagaatataccctgatgggtacggatggccatccgtttggttggccgagcaatggtttcccgggtccgcagggtccgtattactgcggtgtcggcgcagatcgtgcttacggtcgcgacattgtggaagcacactatcgtgcttgtctgtacgcgggtgttaaaatcgccggcaccaatgcagaagtcatgccggctcagtgggaatttcaaattggcccgtgcgaaggtatcagcatgggcgatcatctgtgggttgctcgtttcatcctgcaccgcgtctgtgaagattttggtgtgattgcgaccttcgacccgaaaccgatcccgggcaactggaatggtgctggctgccataccaactttagcacgaaagcgatgcgtgaagaaaatggcctgaaatacatcgaagaagcaatcgaaaaactgtctaaacgtcatcagtatcacattcgcgcctacgatccgaaaggcggtctggacaacgcacgtcgcctgaccggttttcacgaaacgagcaacatcaatgatttctctgcgggcgttgccaatcgctcagcctcgattcgtatcccgcgcaccgtcggtcaagagaaaaaaggctattttgaagatcgtcgcccgagtgcaaactgtgacccgttctccgtgacggaagccctgatccgcacctgtctgctgaatgaaaccggcgatgaaccgttccaatacaaaaat

SEQ ID NO: 6 - protein, 445 aa, Lactobacillus acidophilus
MSKQYTTEEIRKEVADKDVRFLRLCFTDINGTEKAVEVPTSQLDKVLTNDIRFDGSSIDGFVRLEESDMVLYPDFSTWSVLPWGDEHGGKIGRLICSVHMTDGKPFAGDPRNNLKRVLGEMKEAGFDTFDIGFEMEFHLFKLDENGNWTTEVPDHASYFDMTSDDEGARCRREIVETLEEIGFEVEAAHHEVGDGQQEIDFRFDDALTTADRCQTFKMVARHIARKHGLFATFMAKPVEGQAGNGMHNNMSLFKNKHNVFYDKDGEFHLSNTALYFLNGILEHARAITAIGNPTVNSYKRLIPGFEAPVYIAWAAKNRSPLVRIPSAGEINTRLEMRSADPTANPYLLLAACLTAGLKGIKEQKMPMKPVEENIFEMTEEERAEHGIKPLPTTLHNAIKAFKEDDLIKSALGEHLTHSFIESKELEWSKYSQSVSDWERQRYMNW

SEQ ID NO: 7 - protein, 356 aa, Zea mays
MACLTDLVNLNLSDNTEKIIAEYIWIGGSGMDLRSKARTLSGPVTDPSKLPKWNYDGSSTGQAPGEDSEVILYPQAIFKDPFRRGNNILVMCDCYTPAGEPIPTNKRYNAAKIFSSPEVAAEEPWYGIEQEYTLLQKDTNWPLGWPIGGFPGPQGPYYCGIGAEKSFGRDIVDAHYKACLYAGINISGINGEVMPGQWEFQVGPSVGISSGDQVWVARYILERITEIAGVVVTFDPKPIPGDWNGAGAHTNYSTESMRKEGGYEVIKAAIEKLKLRHREHIAAYGEGNERRLTGRHETADINTFSWGVANRGASVRVGRETEQNGKGYFEDRRPASNMDPYVVTSMIAETTIIWKP